European Patent Application EP 4 130 043 A1, published February 8, 2023. Title: ANTI-HUMAN CD47 ANTIBODY AND ANTIGEN-BINDING FRAGMENT THEREOF, AND PREPARATION METHOD THEREFOR AND USE THEREOF. Applicant: SUZHOU ZELGEN BIOPHARMACEUTICALS CO., LTD. SHANGHAI ZELGEN PHARMA.TECH CO., LTD. The sequence listing filed with the application follows.

SEQUENCE LISTING (18 sequences)

SEQ ID NO: 1 - protein, 10 aa, Artificial sequence
  heavy chain complementarity determining region VH CDR1
GFTFSDYGMA

SEQ ID NO: 2 - protein, 17 aa, Artificial sequence
  heavy chain complementarity determining region VH CDR2
FITNLASSIYYADTVTG

SEQ ID NO: 3 - protein, 11 aa, Artificial sequence
  heavy chain complementarity determining region VH CDR3
ARAGDYRSFPY

SEQ ID NO: 4 - protein, 10 aa, Artificial sequence
  light chain complementarity determining region VL CDR1
SASSSVNYVN

SEQ ID NO: 5 - protein, 7 aa, Artificial sequence
  light chain complementarity determining region VL CDR2
GISNLAS

SEQ ID NO: 6 - protein, 8 aa, Artificial sequence
  light chain complementarity determining region VL CDR3
QQRSTFPP

SEQ ID NO: 7 - protein, 118 aa, Artificial sequence
  Heavy chain variable region of the human-mouse chimeric antibody UM03-L4
EVKLVESGGDLVQPGGSRKLSCAASGFTFSDYGMAWIRQAPGKGPEWIAFITNLASSIYYADTVTGRFTISRENAKNTLYLEMSSLRSEDTAMYYCARAGDYRSFPYWGQGTPVTVSA

SEQ ID NO: 8 - protein, 107 aa, Artificial sequence
  Light chain variable region of the human-mouse chimeric antibody UM03-L4
EILLTQSPAIIAASPGEKVTITCSASSSVNYVNWYQQKPGSSPKIWIYGISNLASGVPARFSGSGSGTSFSFTINSMEAEDVATYYCQQRSTFPPYTFGGGTKLEIK

SEQ ID NO: 9 - protein, 445 aa, Artificial sequence
  Heavy chain variable region of human-mouse chimeric antibody UM03-L4
EVKLVESGGDLVQPGGSRKLSCAASGFTFSDYGMAWIRQAPGKGPEWIAFITNLASSIYYADTVTGRFTISRENAKNTLYLEMSSLRSEDTAMYYCARAGDYRSFPYWGQGTPVTVSAASTKGPSVFPLAPCSRSTSESTAALGCLVKDYFPEPVTVSWNSGALTSGVHTFPAVLQSSGLYSLSSVVTVPSSSLGTKTYTCNVDHKPSNTKVDKRVESKYGPPCPPCPAPEFLGGPSVFLFPPKPKDTLMISRTPEVTCVVVDVSQEDPEVQFNWYVDGVEVHNAKTKPREEQFNSTYRVVSVLTVLHQDWLNGKEYKCKVSNKGLPSSIEKTISKAKGQPREPQVYTLPPSQEEMTKNQVSLTCLVKGFYPSDIAVEWESNGQPENNYKTTPPVLDSDGSFFLYSRLTVDKSRWQEGNVFSCSVMHEALHNHYTQKSLSLSLGK

SEQ ID NO: 10 - protein, 214 aa, Artificial sequence
  Light chain variable region of human-mouse chimeric antibody UM03-L4
EILLTQSPAIIAASPGEKVTITCSASSSVNYVNWYQQKPGSSPKIWIYGISNLASGVPARFSGSGSGTSFSFTINSMEAEDVATYYCQQRSTFPPYTFGGGTKLEIKRTVAAPSVFIFPPSDEQLKSGTASVVCLLNNFYPREAKVQWKVDNALQSGNSQESVTEQDSKDSTYSLSSTLTLSKADYEKHKVYACEVTHQGLSSPVTKSFNRGEC

SEQ ID NO: 11 - DNA, 1335 bp, Artificial sequence
  The cDNA sequence encoding the UM03-L4 heavy chain
gaggtgaagctggtggagagcggcggcgacctggtgcagccaggaggatccagaaagctgagctgtgccgccagcggcttcacattcagcgactacggcatggcctggatcaggcaggcccctggcaagggccccgagtggatcgccttcatcaccaatctggcctcctccatctactacgccgacacagtgaccggcaggttcaccatcagcagagagaacgccaagaacacactgtacctggagatgtcctccctgagaagcgaggacacagccatgtactactgtgccagagccggcgactacaggagcttcccctactggggccagggcacacctgtgaccgtgtccgccgctagcacaaagggccccagcgtgtttcctctggccccctgcagcagaagcaccagcgagtccaccgccgccctgggatgcctggtgaaggactacttccctgagcccgtgacagtgagctggaatagcggcgccctgacaagcggcgtgcacacctttcctgccgtgctgcagtccagcggcctgtacagcctgagcagcgtggtgacagtgcctagctcctccctgggcacaaagacatacacctgcaatgtggaccacaagcccagcaacacaaaggtggacaagagagtggagagcaagtacggccctccttgtcccccttgtcctgcccctgagtttctgggcggcccctccgtgtttctgtttcctcccaagcctaaggataccctgatgatctccagaacccccgaggtgacctgtgtggtggtggatgtgagccaggaggaccccgaggtgcagttcaactggtacgtggacggcgtggaggtgcacaatgccaagaccaagcccagggaggagcagtttaactccacatacagggtggtgtccgtgctgaccgtgctgcaccaggactggctgaatggcaaggagtacaagtgtaaggtgagcaacaagggcctgcctagctccatcgagaagaccatctccaaggccaagggccagcctagggagccccaggtgtacacactgcctcccagccaggaggagatgacaaagaaccaggtgagcctgacatgcctggtgaaaggcttctacccttccgacatcgccgtggagtgggagtccaacggccagcctgagaacaattacaagacaaccccccccgtgctggattccgacggcagctttttcctgtactccagactgaccgtggacaagagcagatggcaggagggcaatgtgtttagctgttccgtgatgcacgaggccctgcacaatcactacacacagaagtccctgagcctgagcctgggcaaa

SEQ ID NO: 12 - DNA, 642 bp, Artificial sequence
  The cDNA sequence encoding the light chain UM03-L4
gagatcctgctgacccagagccccgccatcatcgccgccagccctggagagaaggtgaccatcacatgttccgccagcagcagcgtgaattacgtgaactggtatcaacagaagcctggcagcagccctaagatctggatctacggcatctccaacctggcctccggcgtgcctgccaggttcagcggaagcggcagcggcaccagcttcagcttcacaatcaatagcatggaggccgaggatgtggccacatactactgtcagcagagatccacattccctccctacacattcggcggcggcaccaagctggagatcaagcgtacggtggctgcaccatctgtcttcatcttcccgccatctgatgagcagttgaaatctggaactgcctctgttgtgtgcctgctgaataacttctatcccagagaggccaaagtacagtggaaggtggataacgccctccaatcgggtaactcccaggagagtgtcacagagcaggacagcaaggacagcacctacagcctcagcagcaccctgacgctgagcaaagcagactacgagaaacacaaagtctacgcctgcgaagtcacccatcagggcctgagttcgcccgtcacaaagagcttcaacaggggagagtgt

SEQ ID NO: 13 - protein, 118 aa, Artificial sequence
  Heavy chain variable region of humanized antibody UM03-C4
QVQLVESGGGVVQPGGSLRLSCAASGFTFSDYGMAWIRQAPGKGPEWIAFITNLASSIYYADTVTGRFTISRDNSKNTLYLQMNSLRAEDTAVYYCARAGDYRSFPYWGQGTLVTVSA

SEQ ID NO: 14 - protein, 107 aa, Artificial sequence
  Light chain variable region of humanized antibody UM03-C4
EIVLTQSPATLSLSPGERATLSCSASSSVNYVNWYQQKPGQAPRILIYGISNLASGVPARFSGSGSGTDFTLTISSLEPEDFAVYYCQQRSTFPPYTFGQGTKLEIK

SEQ ID NO: 15 - protein, 445 aa, Artificial sequence
  Heavy chain variable region of humanized antibody UM03-C4
QVQLVESGGGVVQPGGSLRLSCAASGFTFSDYGMAWIRQAPGKGPEWIAFITNLASSIYYADTVTGRFTISRDNSKNTLYLQMNSLRAEDTAVYYCARAGDYRSFPYWGQGTLVTVSAASTKGPSVFPLAPCSRSTSESTAALGCLVKDYFPEPVTVSWNSGALTSGVHTFPAVLQSSGLYSLSSVVTVPSSSLGTKTYTCNVDHKPSNTKVDKRVESKYGPPCPPCPAPEFLGGPSVFLFPPKPKDTLMISRTPEVTCVVVDVSQEDPEVQFNWYVDGVEVHNAKTKPREEQFNSTYRVVSVLTVLHQDWLNGKEYKCKVSNKGLPSSIEKTISKAKGQPREPQVYTLPPSQEEMTKNQVSLTCLVKGFYPSDIAVEWESNGQPENNYKTTPPVLDSDGSFFLYSRLTVDKSRWQEGNVFSCSVMHEALHNHYTQKSLSLSLGK

SEQ ID NO: 16 - protein, 214 aa, Artificial sequence
  Light chain variable region of humanized antibody UM03-C4
EIVLTQSPATLSLSPGERATLSCSASSSVNYVNWYQQKPGQAPRILIYGISNLASGVPARFSGSGSGTDFTLTISSLEPEDFAVYYCQQRSTFPPYTFGQGTKLEIKRTVAAPSVFIFPPSDEQLKSGTASVVCLLNNFYPREAKVQWKVDNALQSGNSQESVTEQDSKDSTYSLSSTLTLSKADYEKHKVYACEVTHQGLSSPVTKSFNRGEC

SEQ ID NO: 17 - DNA, 1335 bp, Artificial sequence
  The cDNA sequence encoding the UM03-C4 heavy chain
caggtccagctggtcgagtcaggcggcggcgtcgtgcagcctggaggatcactgagactgagctgcgcagccagcggcttcacattcagcgactacggcatggcctggatcagacaggcacccggcaaagggccagagtggattgctttcatcaccaacctggccagcagcatctactacgccgacaccgtgacaggcagattcaccatcagcagagacaacagcaagaacacactgtacctgcagatgaacagcctgcgcgccgaggacaccgccgtgtactactgcgccagggccggagactacagatcctttccctactgggggcagggaaccctggtgaccgtcagcgccgctagcaccaagggcccatcggtcttccccctggcgccctgctccaggagcacctccgagagcacagccgccctgggctgcctggtcaaggactacttccccgaaccggtgacggtgtcgtggaactcaggcgccctgaccagcggcgtgcacaccttcccggctgtcctacagtcctcaggactctactccctcagcagcgtggtgaccgtgccctccagcagcttgggcacgaagacctacacctgcaacgtagatcacaagcccagcaacaccaaggtggacaagagagttgagtccaaatatggtcccccatgcccaccatgcccagcacctgagttcctggggggaccatcagtcttcctgttccccccaaaacccaaggacactctcatgatctcccggacccctgaggtcacgtgcgtggtggtggacgtgagccaggaagaccccgaggtccagttcaactggtacgtggatggcgtggaggtgcataatgccaagacaaagccgcgggaggagcagttcaacagcacgtaccgtgtggtcagcgtcctcaccgtcctgcaccaggactggctgaacggcaaggagtacaagtgcaaggtctccaacaaaggcctcccgtcctccatcgagaaaaccatctccaaagccaaagggcagccccgagagccacaggtgtacaccctgcccccatcccaggaggagatgaccaagaaccaggtcagcctgacctgcctggtcaaaggcttctaccccagcgacatcgccgtggagtgggagagcaatgggcagccggagaacaactacaagaccacgcctcccgtgctggactccgacggctccttcttcctctacagcaggctaaccgtggacaagagcaggtggcaggaggggaatgtcttctcatgctccgtgatgcatgaggctctgcacaaccactacacacagaagagcctctccctgtctctgggtaaa

SEQ ID NO: 18 - DNA, 642 bp, Artificial sequence
  The cDNA sequence encoding the light chain UM03-C4
gagattgtgctgacccagagccccgccacactgagtctgagtcccggcgagagagcaacactgagttgtagcgccagcagtagtgtgaactacgtgaactggtatcagcagaagcctggacaggctcccagaatcctgatctacggcatctccaacctggccagcggagtgcccgccagattcagcggaagtggcagcgggacagacttcaccctgaccatcagcagcctggaacccgaggatttcgccgtgtactactgccagcagagaagcaccttccccccctatacatttggccagggaaccaagctggaaatcaaacgtacggtggctgcaccatctgtcttcatcttcccgccatctgatgagcagttgaaatctggaactgcctctgttgtgtgcctgctgaataacttctatcccagagaggccaaagtacagtggaaggtggataacgccctccaatcgggtaactcccaggagagtgtcacagagcaggacagcaaggacagcacctacagcctcagcagcaccctgacgctgagcaaagcagactacgagaaacacaaagtctacgcctgcgaagtcacccatcagggcctgagttcgcccgtcacaaagagcttcaacaggggagagtgt